European Patent Application EP 4 356 918 A1, published April 24, 2024. Title: Use for combination therapy in preventing and treating metabolic disease of Lactobacillus fermentum strain and regulatory T cells. Applicant: GI Cell, Inc. The sequence listing filed with the application follows.

SEQUENCE LISTING (2 sequences)

SEQ ID NO: 1 - DNA, 1441 bp, Artificial Sequence
  GB102_16S_full
gcaagtcgaacgcgttggcccaattgattgatggtgcttgcacctgattgattttggtcgccaacgagtggcggacgggtgagtaacacgtaggtaacctgcccagaagcgggggacaacatttggaaacagatgctaataccgcataacaacgttgttcgcatgaacaacgcttaaaagatggcttctcgctatcacttctggatggacctgcggtgcattagcttgttggtggggtaatggcctaccaaggcgatgatgcatagccgagttgagagactgatcggccacaatgggactgagacacggcccatactcctacgggaggcagcagtagggaatcttccacaatgggcgcaagcctgatggagcaacaccgcgtgagtgaagaagggtttcggctcgtaaagctctgttgttaaagaagaacacgtatgagagtaactgttcatacgttgacggtatttaaccagaaagtcacggctaactacgtgccagcagccgcggtaatacgtaggtggcaagcgttatccggatttattgggcgtaaagagagtgcaggcggttttctaagtctgatgtgaaagccttcggcttaaccggagaagtgcatcggaaactggataacttgagtgcagaagagggtagtggaactccatgtgtagcggtggaatgcgtagatatatggaagaacaccagtggcgaaggcggctacctggtctgcaactgacgctgagactcgaaagcatgggtagcgaacaggattagataccctggtagtccatgccgtaaacgatgagtgctaggtgttggagggtttccgcccttcagtgccggagctaacgcattaagcactccgcctggggagtacgaccgcaaggttgaaactcaaaggaattgacgggggcccgcacaagcggtggagcatgtggtttaattcgaagctacgcgaagaaccttaccaggtcttgacatcttgcgccaaccctagagatagggcgtttccttcgggaacgcaatgacaggtggtgcatggtcgtcgtcagctcgtgtcgtgagatgttgggttaagtcccgcaacgagcgcaacccttgttactagttgccagcattaagttgggcactctagtgagactgccggtgacaaaccggaggaaggtggggacgacgtcagatcatcatgccccttatgacctgggctacacacgtgctacaatggacggtacaacgagtcgcgaactcgcgagggcaagcaaatctcttaaaaccgttctcagttcggactgcaggctgcaactcgcctgcacgaagtcggaatcgctagtaatcgcggatcagcatgccgcggtgaatacgttcccgggccttgtacacaccgcccgtcacaccatgagagtttgtaacacccaaagtcggtggggtaaccttttaggagccagcc

SEQ ID NO: 2 - DNA, 1447 bp, Artificial Sequence
  GB103_16S_full
atacatgcaagtcgaacgcgttggcccaattgattgatggtgcttgcacctgattgattttggtcgccaacgagtggcggacgggtgagtaacacgtaggtaacctgcccagaagcgggggacaacatttggaaacagatgctaataccgcataacagcgttgttcgcatgaacaacgcttaaaagatggcttctcgctatcacttctggatggacctgcggtgcattagcttgttggtggggtaacggcctaccaaggcgatgatgcatagccgagttgagagactgatcggccacaatgggactgagacacggcccatactcctacgggaggcagcagtagggaatcttccacaatgggcgcaagcctgatggagcaacaccgcgtgagtgaagaagggtttcggctcgtaaagctctgttgttaaagaagaacacgtatgagagtaactgttcatacgttgacggtatttaaccagaaagtcacggctaactacgtgccagcagccgcggtaatacgtaggtggcaagcgttatccggatttattgggcgtaaagagagtgcaggcggttttctaagtctgatgtgaaagccttcggcttaaccggagaagtgcatcggaaactggataacttgagtgcagaagagggtagtggaactccatgtgtagcggtggaatgcgtagatatatggaagaacaccagtggcgaaggcggctacctggtctgcaactgacgctgagactcgaaagcatgggtagcgaacaggattagataccctggtagtccatgccgtaaacgatgagtgctaggtgttggagggtttccgcccttcagtgccggagctaacgcattaagcactccgcctggggagtacgaccgcaaggttgaaactcaaaggaattgacgggggcccgcacaagcggtggagcatgtggtttaattcgaagctacgcgaagaaccttaccaggtcttgacatcttgcgccaaccctagagatagggcgtttccttcgggaacgcaatgacaggtggtgcatggtcgtcgtcagctcgtgtcgtgagatgttgggttaagtcccgcaacgagcgcaacccttgttactagttgccagcattaagttgggcactctagtgagactgccggtgacaaaccggaggaaggtggggacgacgtcagatcatcatgccccttatgacctgggctacacacgtgctacaatggacggtacaacgagtcgcgaactcgcgagggcaagcaaatctcttaaaaccgttctcagttcggactgcaggctgcaactcgcctgcacgaagtcggaatcgctagtaatcgcggatcagcatgccgcggtgaatacgttcccgggccttgtacacaccgcccgtcacaccatgagagtttgtaacacccaaagtcggtggggtaaccttttaggagccagcc